European Patent Application EP 4 516 811 A2, published March 5, 2025. Title: Inhibitory anti-factor XII/XIIA monoclonal antibodies and their uses. Applicant: CSL Behring GmbH. Application EP. The sequence listing filed with the application follows.

SEQUENCE LISTING (77 sequences)

SEQ ID NO: 1 - protein, 615 aa, Homo sapiens
MRALLLLGFLLVSLESTLSIPPWEAPKEHKYKAEEHTVVLTVTGEPCHFPFQYHRQLYHKCTHKGRPGPQPWCATTPNFDQDQRWGYCLEPKKVKDHCSKHSPCQKGGTCVNMPSGPHCLCPQHLTGNHCQKEKCFEPQLLRFFHKNEIWYRTEQAAVARCQCKGPDAHCQRLASQACRTNPCLHGGRCLEVEGHRLCHCPVGYTGAFCDVDTKASCYDGRGLSYRGLARTTLSGAPCQPWASEATYRNVTAEQARNWGLGGHAFCRNPDNDIRPWCFVLNRDRLSWEYCDLAQCQTPTQAAPPTPVSPRLHVPLMPAQPAPPKPQPTTRTPPQSQTPGALPAKREQPPSLTRNGPLSCGQRLRKSLSSMTRVVGGLVALRGAHPYIAALYWGHSFCAGSLIAPCWVLTAAHCLQDRPAPEDLTVVLGQERRNHSCEPCQTLAVRSYRLHEAFSPVSYQHDLALLRLQEDADGSCALLSPYVQPVCLPSGAARPSETTLCQVAGWGHQFEGAEEYASFLQEAQVPFLSLERCSAPDVHGSSILPGMLCAGFLEGGTDACQGDSGGPLVCEDQAAERRLTLQGIISWGSGCGDRNKPGVYTDVAYYLAWIREHTVS

SEQ ID NO: 2 - protein, 597 aa, Mus musculus
MTALLFLGSLLMSLDLTLSAPPWKDSKKFKDAPDGPTVVLTVDGRLCHFPFQYHRQLHHKCIHKRRPGSRPWCATTPNFDEDQQWGYCLEPKKVKDHCSKHNPCHKGGTCINTPNGPHCLCPEHLTGKHCQKEKCFEPQLLKFFHENELWFRTGPGGVARCECKGSEAHCKPVASQACSINPCLNGGSCLLVEDHPLCRCPTGYTGYFCDLDLWATCYEGRGLSYRGQAGTTQSGAPCQRWTVEATYRNMTEKQALSWGLGHHAFCRNPDNDTRPWCFVWSGDRLSWDYCGLEQCQTPTFAPLVVPESQEESPSQAPSLSHAPNDSTDHQTSLSKTNTMGCGQRFRKGLSSFMRVVGGLVALPGSHPYIAALYWGNNFCAGSLIAPCWVLTAAHCLQNRPAPEELTVVLGQDRHNQSCEWCQTLAVRSYRLHEGFSSITYQHDLALLRLQESKTNSCAILSPHVQPVCLPSGAAPPSETVLCEVAGWGHQFEGAEEYSTFLQEAQVPFIALDRCSNSNVHGDAILPGMLCAGFLEGGTDACQGDSGGPLVCEEGTAEHQLTLRGVISWGSGCGDRNKPGVYTDVANYLAWIQKHIAS

SEQ ID NO: 3 - protein, 595 aa, Rattus norvegicus
MTALLFLGSLLMSLDLTLSAPPWKSKEFKDGAGDPSVVLTVDGKLCHFPFQYHRRLYHKCIHKGQPGSRPWCATTPNFDEDQQWGYCLEPKKVKDHCSKHSPCHKGGTCVNTPNGPHCLCPEHLTGKHCQREKCFESQLLKFFHENEIWFRTGPGGVARCQCKGPQAVCKLLTSQVCRVNPCLNGGTCLLVEDHRLCHCPAGYAGPFCDLDLKATCYEDRGLSYRGQAKTTLSGAPCQRWASEATYRNMTETQALSWGLGHHAFCRNPDNDTRPWCYVWSGDRLSWDYCDLEQCQMPTLTSPVSPESHDMLKPRPPILQSSPRDSTRNQNVVSRTSTVVCGQRFRKRLSSLRRVVGGLVALPGSHPYIAALYWGDSFCAGSLIDPCWVLTAAHCLQKRPAPEELTVVLGQDRHNQSCERCQTLAVHSYRLHEGFSSKTYQHDLALLRLRGRKNSCAILSPHVQPVCLPSSAAPPSETVLCEVAGWGHQFEGAEEYATFLQEAQVPFISLDRCSSSNVHGDAILPGMLCAGFLEGGADACQGDSGGPLVCDEGVTERQLTLRGVISWGSGCGDRNKPGVYTDVANYLDWIQEHTAF

SEQ ID NO: 4 - protein, 129 aa, Homo sapiens
EVQLLESGGGLVQPGGSLRLSCAASGFTFSKYIMQWVRQAPGKGLEWVSGIRPSGGTTVYADSVKGRFTISRDNSKNTLYLQMNSLRAEDTAVYYCARALPRSGYLISPHYYYYALDVWGQGTTVTVSS

SEQ ID NO: 5 - protein, 110 aa, Homo sapiens
QSELTQPPSASGTPGQRVTISCSGSSSNIGRNYVYWYQQVPGTAPKLLIYSNNQRPSGVPDRFSGSKSGTSASLVISGLRSEDEADYYCAAWDASLRGVFGGGTKLTVLG

SEQ ID NO: 6 - protein, 5 aa, Homo sapiens
KYIMQ

SEQ ID NO: 7 - protein, 17 aa, Homo sapiens
GIRPSGGTTVYADSVKG

SEQ ID NO: 8 - protein, 17 aa, synthetic construct
  REGION 1..17: note = Heavy chain CDR2 showing variations
  SITE 3: note = V-segment - X is selected from Arg, Asn, and Asp
  SITE 4: note = V-segment - X is selected from Pro, Val, Ile and Met
  SITE 5: note = V-segment - X is selected from Ser, Pro and Ala
  SITE 6: note = V-segment - X is selected from Gly, Leu, Val and Thr
  SITE 7: note = V-segment - X is selected from Gly, Tyr, Gln, Lys, Arg, Asn and Met
  SITE 8: note = V-segment - X is selected from Thr, Gly and Ser
GIXXXXXXTVYADSVKG

SEQ ID NO: 9 - protein, 20 aa, Homo sapiens
ALPRSGYLISPHYYYYALDV

SEQ ID NO: 10 - protein, 20 aa, synthetic construct
  REGION 1..20: note = Heavy chain CDR3 showing variations
  SITE 9: note = V-segment - X is selected from Ala, Met and Val
  SITE 10: note = V-segment - X is selcted from Ser and Lys
  SITE 11: note = V-segment - X is selected from Pro, Lys, Thr and His
  SITE 12: note = V-segment - X is selected from His, Asn, Gly and Gln
ALPRSGYLXXXXYYYYALDV

SEQ ID NO: 11 - protein, 13 aa, Homo sapiens
SGSSSNIGRNYVY

SEQ ID NO: 12 - protein, 7 aa, Homo sapiens
SNNQRPS

SEQ ID NO: 13 - protein, 10 aa, Homo sapiens
AAWDASLRGV

SEQ ID NO: 14 - skipped

SEQ ID NO: 15 - protein, 124 aa, synthetic construct
  REGION 1..124: note = stop template to generate diverse antibodies
  REGION 30..35: note = misc_feature - X can be any naturally occurring amino acid (except Cys)
EVQLLESGGGLVQPGGSLRLSCAASGFTFXXXXXXWVRQAPGKGLEWVSGIRPSGGTTVYADSVKGRFTISRDNSKNTLYLQMNSLRAEDTAVYYCARALPRSGYLISPHYYYYALDVWGQGTT

SEQ ID NO: 16 - DNA, 53 bp, synthetic construct
  misc_feature 1..53: note = Mutagenic trimer mix
  misc_feature 20..37: note = n is a, c, g, or t
  source 1..53: mol_type = other DNA
agcaagcggttttacctttnnnnnnnnnnnnnnnnnntgggttcgccaggcac

SEQ ID NO: 17 - protein, 133 aa, synthetic construct
  REGION 1..133: note = stop template to generate diverse antibodies
  REGION 52..57: note = misc_feature - X can be any naturally occurring amino acid (except Cys)
EVQLLESGGGLVQPGGSLRLSCAASGFTFSKYIMQWVRQAPGKGLEWVSGIXXXXXXTVYADSVKGRFTISRDNSKNTLYLQMNSLRAEDTAVYYCARALPRSGYLISPHYYYYALDVWGQGTTVTVSSASTK

SEQ ID NO: 18 - DNA, 56 bp, synthetic construct
  misc_feature 1..56: note = Mutagenic trimer mix
  misc_feature 20..37: note = n is a, c, g, or t
  source 1..56: mol_type = other DNA
ggaatgggttagcggtattnnnnnnnnnnnnnnnnnnaccgtttatgcagatagcg

SEQ ID NO: 19 - protein, 133 aa, synthetic construct
  REGION 1..133: note = stop template to generate diverse antibodies
  REGION 100..105: note = misc_feature - X can be any naturally occurring amino acid (except Cys)
EVQLLESGGGLVQPGGSLRLSCAASGFTFSKYIMQWVRQAPGKGLEWVSGIRPSGGTTVYADSVKGRFTISRDNSKNTLYLQMNSLRAEDTAVYYCARAXXXXXXLISPHYYYYALDVWGQGTTVTVSSASTK

SEQ ID NO: 20 - DNA, 57 bp, synthetic construct
  misc_feature 1..57: note = Mutagenic trimer mix
  misc_feature 20..37: note = n is a, c, g, or t
  source 1..57: mol_type = other DNA
ttattattgcgcacgtgcannnnnnnnnnnnnnnnnnctgatttctccgcattatta

SEQ ID NO: 21 - protein, 133 aa, synthetic construct
  REGION 1..133: note = stop template to generate diverse antibodies
  REGION 105..110: note = misc_feature - X can be any naturally occurring amino acid (except Cys)
EVQLLESGGGLVQPGGSLRLSCAASGFTFSKYIMQWVRQAPGKGLEWVSGIRPSGGTTVYADSVKGRFTISRDNSKNTLYLQMNSLRAEDTAVYYCARALPRSGXXXXXXYYYYALDVWGQGTTVTVSSASTK

SEQ ID NO: 22 - DNA, 56 bp, synthetic construct
  misc_feature 1..56: note = Mutagenic trimer mix
  misc_feature 18..35: note = n is a, c, g, or t
  source 1..56: mol_type = other DNA
cactgcctcgtagcggtnnnnnnnnnnnnnnnnnntattattattatgccctggat

SEQ ID NO: 23 - protein, 120 aa, synthetic construct
  REGION 1..120: note = stop template to generate diverse antibodies
  REGION 27..32: note = misc_feature - X can be any naturally occurring amino acid (except Cys)
QSVLTQPPSASGTPGQRVTISCSGSSXXXXXXYVYWYQQLPGTAPKLLIYSNNQRPSGVPDRFSGSKSGTSASLAISGLRSEDEADYYCAAWDASLRGVFGGGTKLTVLGQPKAAPSVTL

SEQ ID NO: 24 - DNA, 55 bp, synthetic construct
  misc_feature 1..55: note = Mutagenic trimer mix
  misc_feature 18..35: note = n is a, c, g, or t
  source 1..55: mol_type = other DNA
gctgtagcggtagcagcnnnnnnnnnnnnnnnnnntatgtgtattggtatcagca

SEQ ID NO: 25 - protein, 120 aa, synthetic construct
  REGION 1..120: note = stop template to generate diverse antibodies
  REGION 90..95: note = misc_feature - X can be any naturally occurring amino acid (except Cys)
QSVLTQPPSASGTPGQRVTISCSGSSSNIGRNYVYWYQQLPGTAPKLLIYSNNQRPSGVPDRFSGSKSGTSASLAISGLRSEDEADYYCXXXXXXLRGVFGGGTKLTVLGQPKAAPSVTL

SEQ ID NO: 26 - DNA, 57 bp, synthetic construct
  misc_feature 1..57: note = Mutagenic trimer mix
  misc_feature 22..39: note = n is a, c, g, or t
  source 1..57: mol_type = other DNA
gatgaagccgattattattgtnnnnnnnnnnnnnnnnnnctgcgtggtgtttttggt

SEQ ID NO: 27 - protein, 120 aa, synthetic construct
  REGION 1..120: note = stop template to generate diverse antibodies
  REGION 94..99: note = misc_feature - X can be any naturally occurring amino acid (except Cys)
QSVLTQPPSASGTPGQRVTISCSGSSSNIGRNYVYWYQQLPGTAPKLLIYSNNQRPSGVPDRFSGSKSGTSASLAISGLRSEDEADYYCAAWDXXXXXXFGGGTKLTVLGQPKAAPSVTL

SEQ ID NO: 28 - DNA, 55 bp, synthetic construct
  misc_feature 1..55: note = Mutagenic trimer mix
  misc_feature 20..37: note = n is a, c, g, or t
  source 1..55: mol_type = other DNA
ttattgtgcagcatgggatnnnnnnnnnnnnnnnnnntttggtggtggcaccaaa

SEQ ID NO: 29 - protein, 17 aa, synthetic construct
  REGION 1..17: note = Affinity-matured HCDR2
GINVPLYGTVYADSVKG

SEQ ID NO: 30 - protein, 17 aa, synthetic construct
  REGION 1..17: note = Affinity-matured HCDR2
GINVPVQGTVYADSVKG

SEQ ID NO: 31 - protein, 17 aa, synthetic construct
  REGION 1..17: note = Affinity-matured HCDR2
GIDIPTKGTVYADSVKG

SEQ ID NO: 32 - protein, 17 aa, synthetic construct
  REGION 1..17: note = Affinity-matured HCDR2
GIDMPTKGTVYADSVKG

SEQ ID NO: 33 - protein, 17 aa, synthetic construct
  REGION 1..17: note = Affinity-matured HCDR2
GINPATRTTVYADSVKG

SEQ ID NO: 34 - protein, 17 aa, synthetic construct
  REGION 1..17: note = Affinity-matured HCDR2
GINPATKTTVYADSVKG

SEQ ID NO: 35 - protein, 17 aa, synthetic construct
  REGION 1..17: note = Affinity-matured HCDR2
GIDVPVRGTVYADSVKG

SEQ ID NO: 36 - protein, 17 aa, synthetic construct
  REGION 1..17: note = Affinity-matured HCDR2
GINPATRSTVYADSVKG

SEQ ID NO: 37 - protein, 17 aa, synthetic construct
  REGION 1..17: note = Affinity-matured HCDR2
GINPATNTTVYADSVKG

SEQ ID NO: 38 - protein, 17 aa, synthetic construct
  REGION 1..17: note = Affinity-matured HCDR2
GINPATMTTVYADSVKG

SEQ ID NO: 39 - protein, 20 aa, synthetic construct
  REGION 1..20: note = Affinity-matured HCDR3
ALPRSGYLMKKNYYYYALDV

SEQ ID NO: 40 - protein, 20 aa, synthetic construct
  REGION 1..20: note = Affinity-matured HCDR3
ALPRSGYLMKTGYYYYALDV

SEQ ID NO: 41 - protein, 20 aa, synthetic construct
  REGION 1..20: note = Affinity-matured HCDR3
ALPRSGYLVKKQYYYYALDV

SEQ ID NO: 42 - protein, 20 aa, synthetic construct
  REGION 1..20: note = Affinity-matured HCDR3
ALPRSGYLVKHGYYYYALDV

SEQ ID NO: 43 - protein, 20 aa, synthetic construct
  REGION 1..20: note = Affinity-matured HCDR3
ALPRSGYLMKPGYYYYALDV

SEQ ID NO: 44 - protein, 13 aa, synthetic construct
  REGION 1..13: note = Affinity-matured LCDR1
SGSSEMTVHHYVY

SEQ ID NO: 45 - protein, 13 aa, synthetic construct
  REGION 1..13: note = Affinity-matured LCDR1
SGSSFSHPHHYVY

SEQ ID NO: 46 - protein, 13 aa, synthetic construct
  REGION 1..13: note = Affinity-matured LCDR1
SGSSEFVEYNYVY

SEQ ID NO: 47 - protein, 13 aa, synthetic construct
  REGION 1..13: note = Affinity-matured LCDR1
SGSSDTNSHHYVY

SEQ ID NO: 48 - protein, 13 aa, synthetic construct
  REGION 1..13: note = Affinity-matured LCDR1
SGSSWTEQHNYVY

SEQ ID NO: 49 - protein, 13 aa, synthetic construct
  REGION 1..13: note = Affinity-matured LCDR1
SGSSVMVTNHYVY

SEQ ID NO: 50 - protein, 13 aa, synthetic construct
  REGION 1..13: note = Affinity-matured LCDR1
SGSSGMVEQNYVY

SEQ ID NO: 51 - protein, 13 aa, synthetic construct
  REGION 1..13: note = Affinity-matured LCDR1
SGSSFKVEETYVY

SEQ ID NO: 52 - protein, 10 aa, synthetic construct
  REGION 1..10: note = Affinity-matured LCDR3
ASWYNDLRGV

SEQ ID NO: 53 - protein, 10 aa, synthetic construct
  REGION 1..10: note = Affinity-matured LCDR3
ASWEIPLRGV

SEQ ID NO: 54 - protein, 10 aa, synthetic construct
  REGION 1..10: note = Affinity-matured LCDR3
ASWTNELRGV

SEQ ID NO: 55 - protein, 10 aa, synthetic construct
  REGION 1..10: note = Affinity-matured LCDR3
ASWWNDLRGV

SEQ ID NO: 56 - protein, 10 aa, synthetic construct
  REGION 1..10: note = Affinity-matured LCDR3
ASWELPLRGV

SEQ ID NO: 57 - protein, 10 aa, synthetic construct
  REGION 1..10: note = Affinity-matured LCDR3
ASWSIPLRGV

SEQ ID NO: 58 - protein, 10 aa, synthetic construct
  REGION 1..10: note = Affinity-matured LCDR3
ASWEVPLRGV

SEQ ID NO: 59 - protein, 10 aa, synthetic construct
  REGION 1..10: note = Affinity-matured LCDR3
AAWDPQVRLA

SEQ ID NO: 60 - protein, 10 aa, synthetic construct
  REGION 1..10: note = Affinity-matured LCDR3
AAWDQQVRLD

SEQ ID NO: 61 - protein, 10 aa, synthetic construct
  REGION 1..10: note = Affinity-matured LCDR3
AAWDQQVRKT

SEQ ID NO: 62 - protein, 10 aa, synthetic construct
  REGION 1..10: note = Affinity-matured LCDR3
AAWDERVRLM

SEQ ID NO: 63 - protein, 10 aa, synthetic construct
  REGION 1..10: note = Affinity-matured LCDR3
AAWDNQVRLG

SEQ ID NO: 64 - DNA, 21 bp, synthetic construct
  misc_feature 1..21: note = Sequencing primer
  source 1..21: mol_type = other DNA
gtccttgaccaggcagcccag

SEQ ID NO: 65 - DNA, 21 bp, synthetic construct
  misc_feature 1..21: note = Sequencing primer
  source 1..21: mol_type = other DNA
gtgagttagctcactcattag

SEQ ID NO: 66 - DNA, 21 bp, synthetic construct
  misc_feature 1..21: note = Sequencing primer
  source 1..21: mol_type = other DNA
ttttcatcggcattttcggtc

SEQ ID NO: 67 - DNA, 24 bp, synthetic construct
  misc_feature 1..24: note = Sequencing primer
  source 1..24: mol_type = other DNA
ccatctgatgagcagttgaaatct

SEQ ID NO: 68 - DNA, 24 bp, synthetic construct
  misc_feature 1..24: note = Sequencing primer
  source 1..24: mol_type = other DNA
gttcccgccctcctctgaggagct

SEQ ID NO: 69 - DNA, 23 bp, synthetic construct
  misc_feature 1..23: note = Sequencing primer
  source 1..23: mol_type = other DNA
agcggataacaatttcacacagg

SEQ ID NO: 70 - DNA, 19 bp, synthetic construct
  misc_feature 1..19: note = Sequencing primer
  source 1..19: mol_type = other DNA
ggttctggcaaatattctg

SEQ ID NO: 71 - DNA, 19 bp, synthetic construct
  misc_feature 1..19: note = Sequencing primer
  source 1..19: mol_type = other DNA
gttgcaccgaccgaatgta

SEQ ID NO: 72 - DNA, 25 bp, synthetic construct
  misc_feature 1..25: note = Sequencing primer
  source 1..25: mol_type = other DNA
accgtgagctggaacagcggtgcgc

SEQ ID NO: 73 - protein, 129 aa, synthetic construct
  REGION 1..129: note = Affinity-matured vH region
EVQLLESGGGLVQPGGSLRLSCAASGFTFSKYIMQWVRQAPGKGLEWVSGIDIPTKGTVYADSVKGRFTISRDNSKNTLYLQMNSLRAEDTAVYYCARALPRSGYLISPHYYYYALDVWGQGTTVTVSS

SEQ ID NO: 74 - protein, 129 aa, synthetic construct
  REGION 1..129: note = Affinity-matured vH region
EVQLLESGGGLVQPGGSLRLSCAASGFTFSKYIMQWVRQAPGKGLEWVSGINVPVQGTVYADSVKGRFTISRDNSKNTLYLQMNSLRAEDTAVYYCARALPRSGYLISPHYYYYALDVWGQGTTVTVSS

SEQ ID NO: 75 - protein, 120 aa, synthetic construct
  REGION 1..120: note = Affinity-matured vL region
QSVLTQPPSASGTPGQRVTISCSGSSEMTVHHYVYWYQQLPGTAPKLLIYSNNQRPSGVPDRFSGSKSGTSASLAISGLRSEDEADYYCAAWDASLRGVFGGGTKLTVLGQPKAAPSVTL

SEQ ID NO: 76 - protein, 130 aa, synthetic construct
  REGION 1..130: note = Affinity-matured vH region
EVQLLESGGGLVQPGGSLRLSCAASGFTFSKYIMQWVRQAPGKGLEWVSGIDMPTKGGTVYADSVKGRFTISRDNSKNTLYLQMNSLRAEDTAVYYCARALPRSGYLISPHYYYYALDVWGQGTTVTVSS

SEQ ID NO: 77 - protein, 131 aa, synthetic construct
  REGION 1..131: note = Affinity-matured vH region
EVQLLESGGGLVQPGGSLRLSCAASGFTFSKYIMQWVRQAPGKGLEWVSGINVPLYGGGTVYADSVKGRFTISRDNSKNTLYLQMNSLRAEDTAVYYCARALPRSGYLISPHYYYYALDVWGQGTTVTVSS